European Patent Specification EP 3 891 172 B1, published January 31, 2024. Title: Polypeptide and its use in affinity purification. Applicant: Oxford University Innovation Limited. The sequence listing filed with the application follows.

SEQUENCE LISTING (26 sequences)

SEQ ID NO: 1 - protein, 115 aa, Artificial Sequence
  SpyDock variant
  MISC_FEATURE (79)..(79): X is alanine, glycine, serine, asparagine or threonine
AMVTTLSGLSGEQGPSGDMTTEEDSATHIKFSKRDEDGRELAGATMELRDCSGKTISTWISDGHVKDFYLYPGKYTFVXTAAPDGYEVATPITFTVNEDGQVTVNGEATEGDAHT

SEQ ID NO: 2 - protein, 92 aa, Artificial Sequence
  Portion of SpyDock variant
  MISC_FEATURE (56)..(56): X is alanine, glycine, serine, asparagine or threonine
DSATHIKFSKRDEDGRELAGATMELRDCSGKTISTWISDGHVKDFYLYPGKYTFVXTAAPDGYEVATPITFTVNEDGQVTVNGEATEGDAHT

SEQ ID NO: 3 - protein, 14 aa, Artificial Sequence
  SpyTag 002
VPTIVMVDAYKRYK

SEQ ID NO: 4 - protein, 13 aa, Artificial Sequence
  SpyTag
AHIVMVDAYKPTK

SEQ ID NO: 5 - protein, 16 aa, Artificial Sequence
  SpyTag2.1
RGVPHIVMVDAYKRYK

SEQ ID NO: 6 - protein, 115 aa, Artificial Sequence
  SpyDock
AMVTTLSGLSGEQGPSGDMTTEEDSATHIKFSKRDEDGRELAGATMELRDCSGKTISTWISDGHVKDFYLYPGKYTFVATAAPDGYEVATPITFTVNEDGQVTVNGEATEGDAHT

SEQ ID NO: 7 - protein, 92 aa, Artificial Sequence
  Portion of SpyDock
DSATHIKFSKRDEDGRELAGATMELRDCSGKTISTWISDGHVKDFYLYPGKYTFVATAAPDGYEVATPITFTVNEDGQVTVNGEATEGDAHT

SEQ ID NO: 8 - DNA, 345 bp, Artificial Sequence
  SpyDock DNA
gccatggtaaccaccttatcaggtttatcaggtgagcaaggtccgtccggtgatatgacaactgaagaagatagtgctacccatattaaattctcaaaacgtgatgaggacggccgtgagttagctggtgcaactatggagttgcgtgattgctctggtaaaactattagtacatggatttcagatggacatgtgaaggatttctacctgtatccaggaaaatatacatttgtcgcgaccgcagcaccagacggttatgaggtagcaactccaattacctttacagttaatgaggacggtcaggttactgtaaatggcgaagcaactgaaggtgacgctcatact

SEQ ID NO: 9 - DNA, 276 bp, Artificial Sequence
  Portion of SpyDock DNA
gatagtgctacccatattaaattctcaaaacgtgatgaggacggccgtgagttagctggtgcaactatggagttgcgtgattgctctggtaaaactattagtacatggatttcagatggacatgtgaaggatttctacctgtatccaggaaaatatacatttgtcgcgaccgcagcaccagacggttatgaggtagcaactccaattacctttacagttaatgaggacggtcaggttactgtaaatggcgaagcaactgaaggtgacgctcatact

SEQ ID NO: 10 - protein, 115 aa, Artificial Sequence
  SpyCatcher
AMVDTLSGLSSEQGQSGDMTIEEDSATHIKFSKRDEDGKELAGATMELRDSSGKTISTWISDGQVKDFYLYPGKYTFVETAAPDGYEVATAITFTVNEQGQVTVNGKATKGDAHI

SEQ ID NO: 11 - protein, 115 aa, Artificial Sequence
  SpyCatcher002
AMVTTLSGLSGEQGPSGDMTTEEDSATHIKFSKRDEDGRELAGATMELRDSSGKTISTWISDGHVKDFYLYPGKYTFVETAAPDGYEVATAITFTVNEQGQVTVNGEATKGDAHT

SEQ ID NO: 12 - protein, 115 aa, Artificial Sequence
  SpyCatcher variant
AMVTTLSGLSGEQGPSGDMTTEEDSATHIKFSKRDEDGRELAGATMELRDSSGKTISTWISDGHVKDFYLYPGKYTFVDTAAPDGYEVATPITFTVNEDGQVTVNGEATEGDAHT

SEQ ID NO: 13 - protein, 115 aa, Artificial Sequence
  SpyCatcher variant
AMVTTLSGLSGEQGPSGDMTTEEDSATHIKFSKRDEDGRELAGATMELRDSSGKTISTWISDGHVKDFYLYPGKYTFVATAAPDGYEVATPITFTVNEDGQVTVNGEATEGDAHT

SEQ ID NO: 14 - protein, 115 aa, Artificial Sequence
  SpyCatcher variant
AMVTTLSGLSGEQGPSGDMTTEEDSATHIKFSKRDEDGRELAGATMELRDCSGKTISTWISDGHVKDFYLYPGKYTFVGTAAPDGYEVATPITFTVNEDGQVTVNGEATEGDAHT

SEQ ID NO: 15 - protein, 115 aa, Artificial Sequence
  SpyCatcher variant
AMVTTLSGLSGEQGPSGDMTTEEDSATHIKFSKRDEDGRELAGATMELRDCSGKTISTWISDGHVKDFYLYPGKYTFVNTAAPDGYEVATPITFTVNEDGQVTVNGEATEGDAHT

SEQ ID NO: 16 - protein, 115 aa, Artificial Sequence
  SpyCatcher variant
AMVTTLSGLSGEQGPSGDMTTEEDSATHIKFSKRDEDGRELAGATMELRDCSGKTISTWISDGHVKDFYLYPGKYTFVQTAAPDGYEVATPITFTVNEDGQVTVNGEATEGDAHT

SEQ ID NO: 17 - protein, 115 aa, Artificial Sequence
  SpyCatcher variant
AMVTTLSGLSGEQGPSGDMTTEEDSATHIKFSKRDEDGRELAGATMELRDCSGKTISTWISDGHVKDFYLYPGKYTFVSTAAPDGYEVATPITFTVNEDGQVTVNGEATEGDAHT

SEQ ID NO: 18 - protein, 115 aa, Artificial Sequence
  SpyCatcher variant
AMVTTLSGLSGEQGPSGDMTTEEDSATHIKFSKRDEDGRELAGATMELRDCSGKTISTWISDGHVKDFYLYPGKYTFVTTAAPDGYEVATPITFTVNEDGQVTVNGEATEGDAHT

SEQ ID NO: 19 - protein, 115 aa, Artificial Sequence
  SpyCatcher variant
AMVTTLSGLSGEQGPSGDMTTEEDSATHIKFSKRDEDGRELAGATMELRDCSGKTISTWISDGHVKDFYLYPGKYTFVVTAAPDGYEVATPITFTVNEDGQVTVNGEATEGDAHT

SEQ ID NO: 20 - protein, 115 aa, Artificial Sequence
  SpyCatcher variant
AMVTTLSGLSGEQGPSGDMTTEEDSATHIAFSKRDEDGRELAGATMELRDCSGKTISTWISDGHVKDFYLYPGKYTFVATAAPDGYEVATPITFTVNEDGQVTVNGEATEGDAHT

SEQ ID NO: 21 - protein, 115 aa, Artificial Sequence
  SpyCatcher variant
AMVDTLSGLSSEQGQSGDMTIEEDSATHIKFSKRDEDGKELAGATMELRDCSGKTISTWISDGQVKDFYLYPGKYTFVATAAPDGYEVATAITFTVNEQGQVTVNGKATKGDAHI

SEQ ID NO: 22 - protein, 115 aa, Artificial Sequence
  SpyCatcher variant
AMVTTLSGLSGEQGPSGDMTTEEDSATHIKFSKRDEDGRELAGATMELRDCSGKTISTWISDGHVKDFYLYPGKYTFVATAAPDGYEVATAITFTVNEQGQVTVNGEATKGDAHT

SEQ ID NO: 23 - protein, 115 aa, Artificial Sequence
  SpyCatcher variant
AMVTTLSGLSGEQGPSGDMTTEEDSATHIKFSKRDEDGRELAGATMELRDCSGKTISTWISDGHVKDFYLYPGKYTFVDTAAPDGYEVATPITFTVNEDGQVTVNGEATEGDAHT

SEQ ID NO: 24 - protein, 122 aa, Artificial Sequence
  SpyCatcher variant
DCDIGSGAMVTTLSGLSGEQGPSGDMTTEEDSATHIKFSKRDEDGRELAGATMELRDSSGKTISTWISDGHVKDFYLYPGKYTFVATAAPDGYEVATPITFTVNEDGQVTVNGEATEGDAHT

SEQ ID NO: 25 - protein, 115 aa, Artificial Sequence
  SpyCatcher variant
AMVTTLSGLSGEQGPSGDMTTEEDSATHIKFSKRDEDGRELAGATMELRDSSGKTICTWISDGHVKDFYLYPGKYTFVATAAPDGYEVATPITFTVNEDGQVTVNGEATEGDAHT

SEQ ID NO: 26 - protein, 7 aa, Artificial Sequence
  TEV recognition site
ENLYFQG